European Patent Application EP 4 582 095 A1, published July 9, 2025. Title: 티로시나아제 활성을 촉진하는 펩타이드 및 이의 용도. Applicant: HYSENSBIO CO., LTD. Application KR 10-2022-0109842, filed August 31, 2023. The sequence listing filed with the application follows.

SEQUENCE LISTING (96 sequences)

SEQ ID NO: 1 - protein, 10 aa, synthetic construct
  REGION 1..10: note = Novel peptide
KYQRRKKNKY

SEQ ID NO: 2 - protein, 10 aa, synthetic construct
  REGION 1..10: note = Novel peptide
KYQRRKRNKY

SEQ ID NO: 3 - protein, 10 aa, synthetic construct
  REGION 1..10: note = Novel peptide
KYQRRRKNKY

SEQ ID NO: 4 - protein, 10 aa, synthetic construct
  REGION 1..10: note = Novel peptide
KYQRRRRNKY

SEQ ID NO: 5 - protein, 10 aa, synthetic construct
  REGION 1..10: note = Novel peptide
KYQRKKKNKY

SEQ ID NO: 6 - protein, 10 aa, synthetic construct
  REGION 1..10: note = Novel peptide
KYQRKRKNKY

SEQ ID NO: 7 - protein, 10 aa, synthetic construct
  REGION 1..10: note = Novel peptide
KYQRKKRNKY

SEQ ID NO: 8 - protein, 10 aa, synthetic construct
  REGION 1..10: note = Novel peptide
KYQRKRRNKY

SEQ ID NO: 9 - protein, 10 aa, synthetic construct
  REGION 1..10: note = Novel peptide
KYQRRKKSKY

SEQ ID NO: 10 - protein, 10 aa, synthetic construct
  REGION 1..10: note = Novel peptide
KYQRRKRSKY

SEQ ID NO: 11 - protein, 10 aa, synthetic construct
  REGION 1..10: note = Novel peptide
KYQRRRKSKY

SEQ ID NO: 12 - protein, 10 aa, synthetic construct
  REGION 1..10: note = Novel peptide
KYQRRRRSKY

SEQ ID NO: 13 - protein, 10 aa, synthetic construct
  REGION 1..10: note = Novel peptide
KYQRKKKSKY

SEQ ID NO: 14 - protein, 10 aa, synthetic construct
  REGION 1..10: note = Novel peptide
KYQRKRKSKY

SEQ ID NO: 15 - protein, 10 aa, synthetic construct
  REGION 1..10: note = Novel peptide
KYQRKKRSKY

SEQ ID NO: 16 - protein, 10 aa, synthetic construct
  REGION 1..10: note = Novel peptide
KYQRKRRSKY

SEQ ID NO: 17 - protein, 10 aa, synthetic construct
  REGION 1..10: note = Novel peptide
KYQRRKKNYK

SEQ ID NO: 18 - protein, 10 aa, synthetic construct
  REGION 1..10: note = Novel peptide
KYQRRKRNYK

SEQ ID NO: 19 - protein, 10 aa, synthetic construct
  REGION 1..10: note = Novel peptide
KYQRRRKNYK

SEQ ID NO: 20 - protein, 10 aa, synthetic construct
  REGION 1..10: note = Novel peptide
KYQRRRRNYK

SEQ ID NO: 21 - protein, 10 aa, synthetic construct
  REGION 1..10: note = Novel peptide
KYQRKKKNYK

SEQ ID NO: 22 - protein, 10 aa, synthetic construct
  REGION 1..10: note = Novel peptide
KYQRKRKNYK

SEQ ID NO: 23 - protein, 10 aa, synthetic construct
  REGION 1..10: note = Novel peptide
KYQRKKRNYK

SEQ ID NO: 24 - protein, 10 aa, synthetic construct
  REGION 1..10: note = Novel peptide
KYQRKRRNYK

SEQ ID NO: 25 - protein, 10 aa, synthetic construct
  REGION 1..10: note = Novel peptide
KYQRRKKSYK

SEQ ID NO: 26 - protein, 10 aa, synthetic construct
  REGION 1..10: note = Novel peptide
KYQRRKRSYK

SEQ ID NO: 27 - protein, 10 aa, synthetic construct
  REGION 1..10: note = Novel peptide
KYQRRRKSYK

SEQ ID NO: 28 - protein, 10 aa, synthetic construct
  REGION 1..10: note = Novel peptide
KYQRRRRSYK

SEQ ID NO: 29 - protein, 10 aa, synthetic construct
  REGION 1..10: note = Novel peptide
KYQRKKKSYK

SEQ ID NO: 30 - protein, 10 aa, synthetic construct
  REGION 1..10: note = Novel peptide
KYQRKRKSYK

SEQ ID NO: 31 - protein, 10 aa, synthetic construct
  REGION 1..10: note = Novel peptide
KYQRKKRSYK

SEQ ID NO: 32 - protein, 10 aa, synthetic construct
  REGION 1..10: note = Novel peptide
KYQRKRRSYK

SEQ ID NO: 33 - protein, 10 aa, synthetic construct
  REGION 1..10: note = Novel peptide
KYRQRKKNKY

SEQ ID NO: 34 - protein, 10 aa, synthetic construct
  REGION 1..10: note = Novel peptide
KYRQRKRNKY

SEQ ID NO: 35 - protein, 10 aa, synthetic construct
  REGION 1..10: note = Novel peptide
KYRQRRKNKY

SEQ ID NO: 36 - protein, 10 aa, synthetic construct
  REGION 1..10: note = Novel peptide
KYRQRRRNKY

SEQ ID NO: 37 - protein, 10 aa, synthetic construct
  REGION 1..10: note = Novel peptide
KYRQKKKNKY

SEQ ID NO: 38 - protein, 10 aa, synthetic construct
  REGION 1..10: note = Novel peptide
KYRQKRKNKY

SEQ ID NO: 39 - protein, 10 aa, synthetic construct
  REGION 1..10: note = Novel peptide
KYRQKKRNKY

SEQ ID NO: 40 - protein, 10 aa, synthetic construct
  REGION 1..10: note = Novel peptide
KYRQKRRNKY

SEQ ID NO: 41 - protein, 10 aa, synthetic construct
  REGION 1..10: note = Novel peptide
KYRQRKKSKY

SEQ ID NO: 42 - protein, 10 aa, synthetic construct
  REGION 1..10: note = Novel peptide
KYRQRKRSKY

SEQ ID NO: 43 - protein, 10 aa, synthetic construct
  REGION 1..10: note = Novel peptide
KYRQRRKSKY

SEQ ID NO: 44 - protein, 10 aa, synthetic construct
  REGION 1..10: note = Novel peptide
KYRQRRRSKY

SEQ ID NO: 45 - protein, 10 aa, synthetic construct
  REGION 1..10: note = Novel peptide
KYRQKKKSKY

SEQ ID NO: 46 - protein, 10 aa, synthetic construct
  REGION 1..10: note = Novel peptide
KYRQKRKSKY

SEQ ID NO: 47 - protein, 10 aa, synthetic construct
  REGION 1..10: note = Novel peptide
KYRQKKRSKY

SEQ ID NO: 48 - protein, 10 aa, synthetic construct
  REGION 1..10: note = Novel peptide
KYRQKRRSKY

SEQ ID NO: 49 - protein, 10 aa, synthetic construct
  REGION 1..10: note = Novel peptide
KYRQRKKNYK

SEQ ID NO: 50 - protein, 10 aa, synthetic construct
  REGION 1..10: note = Novel peptide
KYRQRKRNYK

SEQ ID NO: 51 - protein, 10 aa, synthetic construct
  REGION 1..10: note = Novel peptide
KYRQRRKNYK

SEQ ID NO: 52 - protein, 10 aa, synthetic construct
  REGION 1..10: note = Novel peptide
KYRQRRRNYK

SEQ ID NO: 53 - protein, 10 aa, synthetic construct
  REGION 1..10: note = Novel peptide
KYRQKKKNYK

SEQ ID NO: 54 - protein, 10 aa, synthetic construct
  REGION 1..10: note = Novel peptide
KYRQKRKNYK

SEQ ID NO: 55 - protein, 10 aa, synthetic construct
  REGION 1..10: note = Novel peptide
KYRQKKRNYK

SEQ ID NO: 56 - protein, 10 aa, synthetic construct
  REGION 1..10: note = Novel peptide
KYRQKRRNYK

SEQ ID NO: 57 - protein, 10 aa, synthetic construct
  REGION 1..10: note = Novel peptide
KYRQRKKSYK

SEQ ID NO: 58 - protein, 10 aa, synthetic construct
  REGION 1..10: note = Novel peptide
KYRQRKRSYK

SEQ ID NO: 59 - protein, 10 aa, synthetic construct
  REGION 1..10: note = Novel peptide
KYRQRRKSYK

SEQ ID NO: 60 - protein, 10 aa, synthetic construct
  REGION 1..10: note = Novel peptide
KYRQRRRSYK

SEQ ID NO: 61 - protein, 10 aa, synthetic construct
  REGION 1..10: note = Novel peptide
KYRQKKKSYK

SEQ ID NO: 62 - protein, 10 aa, synthetic construct
  REGION 1..10: note = Novel peptide
KYRQKRKSYK

SEQ ID NO: 63 - protein, 10 aa, synthetic construct
  REGION 1..10: note = Novel peptide
KYRQKKRSYK

SEQ ID NO: 64 - protein, 10 aa, synthetic construct
  REGION 1..10: note = Novel peptide
KYRQKRRSYK

SEQ ID NO: 65 - protein, 10 aa, synthetic construct
  REGION 1..10: note = Novel peptide
KYKQRKKNKY

SEQ ID NO: 66 - protein, 10 aa, synthetic construct
  REGION 1..10: note = Novel peptide
KYKQRKRNKY

SEQ ID NO: 67 - protein, 10 aa, synthetic construct
  REGION 1..10: note = Novel peptide
KYKQRRKNKY

SEQ ID NO: 68 - protein, 10 aa, synthetic construct
  REGION 1..10: note = Novel peptide
KYKQRRRNKY

SEQ ID NO: 69 - protein, 10 aa, synthetic construct
  REGION 1..10: note = Novel peptide
KYKQKKKNKY

SEQ ID NO: 70 - protein, 10 aa, synthetic construct
  REGION 1..10: note = Novel peptide
KYKQKRKNKY

SEQ ID NO: 71 - protein, 10 aa, synthetic construct
  REGION 1..10: note = Novel peptide
KYKQKKRNKY

SEQ ID NO: 72 - protein, 10 aa, synthetic construct
  REGION 1..10: note = Novel peptide
KYKQKRRNKY

SEQ ID NO: 73 - protein, 10 aa, synthetic construct
  REGION 1..10: note = Novel peptide
KYKQRKKSKY

SEQ ID NO: 74 - protein, 10 aa, synthetic construct
  REGION 1..10: note = Novel peptide
KYKQRKRSKY

SEQ ID NO: 75 - protein, 10 aa, synthetic construct
  REGION 1..10: note = Novel peptide
KYKQRRKSKY

SEQ ID NO: 76 - protein, 10 aa, synthetic construct
  REGION 1..10: note = Novel peptide
KYKQRRRSKY

SEQ ID NO: 77 - protein, 10 aa, synthetic construct
  REGION 1..10: note = Novel peptide
KYKQKKKSKY

SEQ ID NO: 78 - protein, 10 aa, synthetic construct
  REGION 1..10: note = Novel peptide
KYKQKRKSKY

SEQ ID NO: 79 - protein, 10 aa, synthetic construct
  REGION 1..10: note = Novel peptide
KYKQKKRSKY

SEQ ID NO: 80 - protein, 10 aa, synthetic construct
  REGION 1..10: note = Novel peptide
KYKQKRRSKY

SEQ ID NO: 81 - protein, 10 aa, synthetic construct
  REGION 1..10: note = Novel peptide
KYKQRKKNYK

SEQ ID NO: 82 - protein, 10 aa, synthetic construct
  REGION 1..10: note = Novel peptide
KYKQRKRNYK

SEQ ID NO: 83 - protein, 10 aa, synthetic construct
  REGION 1..10: note = Novel peptide
KYKQRRKNYK

SEQ ID NO: 84 - protein, 10 aa, synthetic construct
  REGION 1..10: note = Novel peptide
KYKQRRRNYK

SEQ ID NO: 85 - protein, 10 aa, synthetic construct
  REGION 1..10: note = Novel peptide
KYKQKKKNYK

SEQ ID NO: 86 - protein, 10 aa, synthetic construct
  REGION 1..10: note = Novel peptide
KYKQKRKNYK

SEQ ID NO: 87 - protein, 10 aa, synthetic construct
  REGION 1..10: note = Novel peptide
KYKQKKRNYK

SEQ ID NO: 88 - protein, 10 aa, synthetic construct
  REGION 1..10: note = Novel peptide
KYKQKRRNYK

SEQ ID NO: 89 - protein, 10 aa, synthetic construct
  REGION 1..10: note = Novel peptide
KYKQRKKSYK

SEQ ID NO: 90 - protein, 10 aa, synthetic construct
  REGION 1..10: note = Novel peptide
KYKQRKRSYK

SEQ ID NO: 91 - protein, 10 aa, synthetic construct
  REGION 1..10: note = Novel peptide
KYKQRRKSYK

SEQ ID NO: 92 - protein, 10 aa, synthetic construct
  REGION 1..10: note = Novel peptide
KYKQRRRSYK

SEQ ID NO: 93 - protein, 10 aa, synthetic construct
  REGION 1..10: note = Novel peptide
KYKQKKKSYK

SEQ ID NO: 94 - protein, 10 aa, synthetic construct
  REGION 1..10: note = Novel peptide
KYKQKRKSYK

SEQ ID NO: 95 - protein, 10 aa, synthetic construct
  REGION 1..10: note = Novel peptide
KYKQKKRSYK

SEQ ID NO: 96 - protein, 10 aa, synthetic construct
  REGION 1..10: note = Novel peptide
KYKQKRRSYK